European Patent Application EP 4 806 991 A1, published September 16, 2026. Title: Microorganism having enhanced activity of acetohydroxy acid synthase large subunit and uses thereof. Applicant: CJ CheilJedang Corporation. The sequence listing filed with the application follows.

SEQUENCE LISTING (21 sequences)

SEQ ID NO: 1 - protein, 626 aa, synthetic construct
  REGION 1..626: note = ilvB (WT) (NCBI Reference Sequence: WP_003861427.1)
MNVAASQQPTPATVASRGRSAAPERMTGAQAIVRSLEELNADIVFGIPGGAVLPVYDPLYSSTKVRHVLVRHEQGAGHAATGYAQVTGRVGVCIATSGPGATNLVTPIADANLDSVPMVAITGQVGSGLLGTDAFQEADIRGITMPVTKHNFMVTDPNDIPQALAEAFHLAITGRPGPVLVDIPKDVQNAELDFVWPPKIDLPGYRPVSTPHARQIEQAVKLIGEAKKPVLYIGGGVIKADAHEELRAFAEYTGIPVVTTLMALGTFPESHELHMGMPGMHGTVSAVGALQRSDLLIAIGSRFDDRVTGDVDTFAPDAKIIHADIDPAEIGKIKQVEVPIVGDAREVLARLLETTKASKAETEDISEWVDYLKGLKARFPRGYDEQPGDLLAPQFVIETLSKEVGPDAIYCAGVGQHQMWAAQFVDFEKPRTWLNSGGLGTMGYAVPAALGAKAGAPDKEVWAIDGDGCFQMTNQELTTAAVEGFPIKIALINNGNLGMVRQWQTLFYEGRYSNTKLRNQGEYMPDFVTLSEGLGCVAIRVTKAEEVLPAIQKAREINDRPVVIDFIVGEDAQVWPMVSAGSSNSDIQYALGLRPFFDGDESAAEDPADIHEAVSDIDAAVESTEA

SEQ ID NO: 2 - DNA, 1881 bp, synthetic construct
  misc_feature 1..1881: note = gene coding ilvB (WT)
  source 1..1881: mol_type = other DNA
gtgaatgtggcagcttctcaacagcccactcccgccacggttgcaagccgtggtcgatccgccgcccctgagcggatgacaggtgcacaggcaattgttcgatcgctcgaggagcttaacgccgacatcgtgttcggtattcctggtggtgcggtgctaccggtgtatgacccgctctattcctccacaaaggtgcgccacgtcctggtgcgccacgagcagggcgcaggccacgcagcaaccggctacgcgcaggttactggacgcgttggcgtctgcattgcaacctctggcccaggcgcaaccaacttggttaccccaatcgctgatgcaaacttggactccgttcccatggttgccatcaccggccaggtcggaagtggcctgctgggtaccgatgctttccaggaagccgatatccgcggcatcaccatgccagtgaccaagcacaacttcatggtcaccgaccccaacgacattccacaggcattggctgaggcattccacctcgcgattactggtcgccctggccctgttctggtggatattcctaaggatgtccaaaacgctgaattggatttcgtctggccaccaaagatcgacctgccaggctaccgcccagtttctactccgcatgctcgacagattgagcaggctgtcaaactgatcggtgaagccaaaaagccagtcctttacattggcggcggcgttatcaaggctgatgcacacgaagaactgcgtgcatttgctgagtacaccggcatcccagttgtcaccaccttgatggcattgggtaccttcccagagtcccacgagctgcacatgggtatgccaggcatgcacggcaccgtgtccgctgttggcgcactgcagcgcagtgacctgctgattgctatcggttcccgcttcgacgaccgcgtcaccggtgacgttgacaccttcgcacctgatgccaagatcattcacgctgacattgatcctgccgaaatcggcaagatcaagcaggttgaggttccaatcgtgggcgatgcccgcgaggttcttgctcgtctgctggaaaccaccaaggcaagcaaggcagagaccgaggacatctccgagtgggttgattacctcaagggcctcaaggcacgtttcccacgtggctacgacgagcagccaggcgatctgctggcaccacagtttgtcattgaaaccctgtccaaggaagttggccccgacgcaatttactgcgccggcgttggccagcaccagatgtgggcagctcagttcgttgactttgaaaagccacgcacctggctcaactctggcggcctgggcaccatgggctacgcagttcctgcggctcttggagcaaaggctggcgcacctgacaaggaagtctgggctatcgacggcgacggctgtttccagatgaccaaccaggaactcaccaccgccgcagttgaaggtttccccattaagatcgcactaatcaacaacggaaacctgggcatggttcgccaatggcagaccctattctatgaaggacggtactcaaatactaaacttcgtaaccagggcgagtacatgcccgactttgttaccctttctgagggacttggctgtgttgccatccgcgtcaccaaagcggaggaagtactgccagccatccaaaaggctcgagagatcaacgaccgcccagtagtcatcgacttcatcgtcggtgaagacgcacaggtatggccaatggtgtctgctggatcatccaactccgatatccagtacgcactcggattgcgcccattctttgatggtgatgaatctgcagcagaagatcctgccgacattcacgaagccgtcagcgacattgatgccgccgttgaatcgaccgaggcataa

SEQ ID NO: 3 - protein, 626 aa, synthetic construct
  REGION 1..626: note = ilvB (H150R)
MNVAASQQPTPATVASRGRSAAPERMTGAQAIVRSLEELNADIVFGIPGGAVLPVYDPLYSSTKVRHVLVRHEQGAGHAATGYAQVTGRVGVCIATSGPGATNLVTPIADANLDSVPMVAITGQVGSGLLGTDAFQEADIRGITMPVTKRNFMVTDPNDIPQALAEAFHLAITGRPGPVLVDIPKDVQNAELDFVWPPKIDLPGYRPVSTPHARQIEQAVKLIGEAKKPVLYIGGGVIKADAHEELRAFAEYTGIPVVTTLMALGTFPESHELHMGMPGMHGTVSAVGALQRSDLLIAIGSRFDDRVTGDVDTFAPDAKIIHADIDPAEIGKIKQVEVPIVGDAREVLARLLETTKASKAETEDISEWVDYLKGLKARFPRGYDEQPGDLLAPQFVIETLSKEVGPDAIYCAGVGQHQMWAAQFVDFEKPRTWLNSGGLGTMGYAVPAALGAKAGAPDKEVWAIDGDGCFQMTNQELTTAAVEGFPIKIALINNGNLGMVRQWQTLFYEGRYSNTKLRNQGEYMPDFVTLSEGLGCVAIRVTKAEEVLPAIQKAREINDRPVVIDFIVGEDAQVWPMVSAGSSNSDIQYALGLRPFFDGDESAAEDPADIHEAVSDIDAAVESTEA

SEQ ID NO: 4 - DNA, 1881 bp, synthetic construct
  misc_feature 1..1881: note = gene coding ilvB (H150R)
  source 1..1881: mol_type = other DNA
gtgaatgtggcagcttctcaacagcccactcccgccacggttgcaagccgtggtcgatccgccgcccctgagcggatgacaggtgcacaggcaattgttcgatcgctcgaggagcttaacgccgacatcgtgttcggtattcctggtggtgcggtgctaccggtgtatgacccgctctattcctccacaaaggtgcgccacgtcctggtgcgccacgagcagggcgcaggccacgcagcaaccggctacgcgcaggttactggacgcgttggcgtctgcattgcaacctctggcccaggcgcaaccaacttggttaccccaatcgctgatgcaaacttggactccgttcccatggttgccatcaccggccaggtcggaagtggcctgctgggtaccgatgctttccaggaagccgatatccgcggcatcaccatgccagtgaccaagcgcaacttcatggtcaccgaccccaacgacattccacaggcattggctgaggcattccacctcgcgattactggtcgccctggccctgttctggtggatattcctaaggatgtccaaaacgctgaattggatttcgtctggccaccaaagatcgacctgccaggctaccgcccagtttctactccgcatgctcgacagattgagcaggctgtcaaactgatcggtgaagccaaaaagccagtcctttacattggcggcggcgttatcaaggctgatgcacacgaagaactgcgtgcatttgctgagtacaccggcatcccagttgtcaccaccttgatggcattgggtaccttcccagagtcccacgagctgcacatgggtatgccaggcatgcacggcaccgtgtccgctgttggcgcactgcagcgcagtgacctgctgattgctatcggttcccgcttcgacgaccgcgtcaccggtgacgttgacaccttcgcacctgatgccaagatcattcacgctgacattgatcctgccgaaatcggcaagatcaagcaggttgaggttccaatcgtgggcgatgcccgcgaggttcttgctcgtctgctggaaaccaccaaggcaagcaaggcagagaccgaggacatctccgagtgggttgattacctcaagggcctcaaggcacgtttcccacgtggctacgacgagcagccaggcgatctgctggcaccacagtttgtcattgaaaccctgtccaaggaagttggccccgacgcaatttactgcgccggcgttggccagcaccagatgtgggcagctcagttcgttgactttgaaaagccacgcacctggctcaactctggcggcctgggcaccatgggctacgcagttcctgcggctcttggagcaaaggctggcgcacctgacaaggaagtctgggctatcgacggcgacggctgtttccagatgaccaaccaggaactcaccaccgccgcagttgaaggtttccccattaagatcgcactaatcaacaacggaaacctgggcatggttcgccaatggcagaccctattctatgaaggacggtactcaaatactaaacttcgtaaccagggcgagtacatgcccgactttgttaccctttctgagggacttggctgtgttgccatccgcgtcaccaaagcggaggaagtactgccagccatccaaaaggctcgagagatcaacgaccgcccagtagtcatcgacttcatcgtcggtgaagacgcacaggtatggccaatggtgtctgctggatcatccaactccgatatccagtacgcactcggattgcgcccattctttgatggtgatgaatctgcagcagaagatcctgccgacattcacgaagccgtcagcgacattgatgccgccgttgaatcgaccgaggcataa

SEQ ID NO: 5 - DNA, 25 bp, synthetic construct
  misc_feature 1..25: note = primer
  source 1..25: mol_type = other DNA
agcaaccggctacgcgcaggttact

SEQ ID NO: 6 - DNA, 24 bp, synthetic construct
  misc_feature 1..24: note = primer
  source 1..24: mol_type = other DNA
aacctcaacctgcttgatcttgcc

SEQ ID NO: 7 - DNA, 41 bp, synthetic construct
  misc_feature 1..41: note = primer
  source 1..41: mol_type = other DNA
cggggatcccccgggaggacggtactcaaatactaaacttc

SEQ ID NO: 8 - DNA, 38 bp, synthetic construct
  misc_feature 1..38: note = primer
  source 1..38: mol_type = other DNA
tgccgagtgtttcggtctttacagacacgagggacacg

SEQ ID NO: 9 - DNA, 31 bp, synthetic construct
  misc_feature 1..31: note = primer
  source 1..31: mol_type = other DNA
tgtctgtaaagaccgaaacactcggcatcaa

SEQ ID NO: 10 - DNA, 41 bp, synthetic construct
  misc_feature 1..41: note = primer
  source 1..41: mol_type = other DNA
cggggatcccccggggacaactacattattattataccaca

SEQ ID NO: 11 - DNA, 18 bp, synthetic construct
  misc_feature 1..18: note = primer
  source 1..18: mol_type = other DNA
ccgcgtcaccaaagcgga

SEQ ID NO: 12 - DNA, 20 bp, synthetic construct
  misc_feature 1..20: note = primer
  source 1..20: mol_type = other DNA
ttagatcttggccggagcca

SEQ ID NO: 13 - protein, 626 aa, synthetic construct
  REGION 1..626: note = ilvB (H150P)
MNVAASQQPTPATVASRGRSAAPERMTGAQAIVRSLEELNADIVFGIPGGAVLPVYDPLYSSTKVRHVLVRHEQGAGHAATGYAQVTGRVGVCIATSGPGATNLVTPIADANLDSVPMVAITGQVGSGLLGTDAFQEADIRGITMPVTKPNFMVTDPNDIPQALAEAFHLAITGRPGPVLVDIPKDVQNAELDFVWPPKIDLPGYRPVSTPHARQIEQAVKLIGEAKKPVLYIGGGVIKADAHEELRAFAEYTGIPVVTTLMALGTFPESHELHMGMPGMHGTVSAVGALQRSDLLIAIGSRFDDRVTGDVDTFAPDAKIIHADIDPAEIGKIKQVEVPIVGDAREVLARLLETTKASKAETEDISEWVDYLKGLKARFPRGYDEQPGDLLAPQFVIETLSKEVGPDAIYCAGVGQHQMWAAQFVDFEKPRTWLNSGGLGTMGYAVPAALGAKAGAPDKEVWAIDGDGCFQMTNQELTTAAVEGFPIKIALINNGNLGMVRQWQTLFYEGRYSNTKLRNQGEYMPDFVTLSEGLGCVAIRVTKAEEVLPAIQKAREINDRPVVIDFIVGEDAQVWPMVSAGSSNSDIQYALGLRPFFDGDESAAEDPADIHEAVSDIDAAVESTEA

SEQ ID NO: 14 - protein, 626 aa, synthetic construct
  REGION 1..626: note = ilvB (H150N)
MNVAASQQPTPATVASRGRSAAPERMTGAQAIVRSLEELNADIVFGIPGGAVLPVYDPLYSSTKVRHVLVRHEQGAGHAATGYAQVTGRVGVCIATSGPGATNLVTPIADANLDSVPMVAITGQVGSGLLGTDAFQEADIRGITMPVTKNNFMVTDPNDIPQALAEAFHLAITGRPGPVLVDIPKDVQNAELDFVWPPKIDLPGYRPVSTPHARQIEQAVKLIGEAKKPVLYIGGGVIKADAHEELRAFAEYTGIPVVTTLMALGTFPESHELHMGMPGMHGTVSAVGALQRSDLLIAIGSRFDDRVTGDVDTFAPDAKIIHADIDPAEIGKIKQVEVPIVGDAREVLARLLETTKASKAETEDISEWVDYLKGLKARFPRGYDEQPGDLLAPQFVIETLSKEVGPDAIYCAGVGQHQMWAAQFVDFEKPRTWLNSGGLGTMGYAVPAALGAKAGAPDKEVWAIDGDGCFQMTNQELTTAAVEGFPIKIALINNGNLGMVRQWQTLFYEGRYSNTKLRNQGEYMPDFVTLSEGLGCVAIRVTKAEEVLPAIQKAREINDRPVVIDFIVGEDAQVWPMVSAGSSNSDIQYALGLRPFFDGDESAAEDPADIHEAVSDIDAAVESTEA

SEQ ID NO: 15 - DNA, 28 bp, synthetic construct
  misc_feature 1..28: note = primer
  source 1..28: mol_type = other DNA
tgaccaagcctaacttcatggtcaccga

SEQ ID NO: 16 - DNA, 28 bp, synthetic construct
  misc_feature 1..28: note = primer
  source 1..28: mol_type = other DNA
atgaagttaggcttggtcactggcatgg

SEQ ID NO: 17 - DNA, 28 bp, synthetic construct
  misc_feature 1..28: note = primer
  source 1..28: mol_type = other DNA
tgaccaagaataacttcatggtcaccga

SEQ ID NO: 18 - DNA, 28 bp, synthetic construct
  misc_feature 1..28: note = primer
  source 1..28: mol_type = other DNA
atgaagttattcttggtcactggcatgg

SEQ ID NO: 19 - DNA, 1881 bp, synthetic construct
  misc_feature 1..1881: note = gene coding ilvB (H150P)
  source 1..1881: mol_type = other DNA
gtgaatgtggcagcttctcaacagcccactcccgccacggttgcaagccgtggtcgatccgccgcccctgagcggatgacaggtgcacaggcaattgttcgatcgctcgaggagcttaacgccgacatcgtgttcggtattcctggtggtgcggtgctaccggtgtatgacccgctctattcctccacaaaggtgcgccacgtcctggtgcgccacgagcagggcgcaggccacgcagcaaccggctacgcgcaggttactggacgcgttggcgtctgcattgcaacctctggcccaggcgcaaccaacttggttaccccaatcgctgatgcaaacttggactccgttcccatggttgccatcaccggccaggtcggaagtggcctgctgggtaccgatgctttccaggaagccgatatccgcggcatcaccatgccagtgaccaagcctaacttcatggtcaccgaccccaacgacattccacaggcattggctgaggcattccacctcgcgattactggtcgccctggccctgttctggtggatattcctaaggatgtccaaaacgctgaattggatttcgtctggccaccaaagatcgacctgccaggctaccgcccagtttctactccgcatgctcgacagattgagcaggctgtcaaactgatcggtgaagccaaaaagccagtcctttacattggcggcggcgttatcaaggctgatgcacacgaagaactgcgtgcatttgctgagtacaccggcatcccagttgtcaccaccttgatggcattgggtaccttcccagagtcccacgagctgcacatgggtatgccaggcatgcacggcaccgtgtccgctgttggcgcactgcagcgcagtgacctgctgattgctatcggttcccgcttcgacgaccgcgtcaccggtgacgttgacaccttcgcacctgatgccaagatcattcacgctgacattgatcctgccgaaatcggcaagatcaagcaggttgaggttccaatcgtgggcgatgcccgcgaggttcttgctcgtctgctggaaaccaccaaggcaagcaaggcagagaccgaggacatctccgagtgggttgattacctcaagggcctcaaggcacgtttcccacgtggctacgacgagcagccaggcgatctgctggcaccacagtttgtcattgaaaccctgtccaaggaagttggccccgacgcaatttactgcgccggcgttggccagcaccagatgtgggcagctcagttcgttgactttgaaaagccacgcacctggctcaactctggcggcctgggcaccatgggctacgcagttcctgcggctcttggagcaaaggctggcgcacctgacaaggaagtctgggctatcgacggcgacggctgtttccagatgaccaaccaggaactcaccaccgccgcagttgaaggtttccccattaagatcgcactaatcaacaacggaaacctgggcatggttcgccaatggcagaccctattctatgaaggacggtactcaaatactaaacttcgtaaccagggcgagtacatgcccgactttgttaccctttctgagggacttggctgtgttgccatccgcgtcaccaaagcggaggaagtactgccagccatccaaaaggctcgagagatcaacgaccgcccagtagtcatcgacttcatcgtcggtgaagacgcacaggtatggccaatggtgtctgctggatcatccaactccgatatccagtacgcactcggattgcgcccattctttgatggtgatgaatctgcagcagaagatcctgccgacattcacgaagccgtcagcgacattgatgccgccgttgaatcgaccgaggcataa

SEQ ID NO: 20 - DNA, 1881 bp, synthetic construct
  misc_feature 1..1881: note = gene coding ilvB (H150N)
  source 1..1881: mol_type = other DNA
gtgaatgtggcagcttctcaacagcccactcccgccacggttgcaagccgtggtcgatccgccgcccctgagcggatgacaggtgcacaggcaattgttcgatcgctcgaggagcttaacgccgacatcgtgttcggtattcctggtggtgcggtgctaccggtgtatgacccgctctattcctccacaaaggtgcgccacgtcctggtgcgccacgagcagggcgcaggccacgcagcaaccggctacgcgcaggttactggacgcgttggcgtctgcattgcaacctctggcccaggcgcaaccaacttggttaccccaatcgctgatgcaaacttggactccgttcccatggttgccatcaccggccaggtcggaagtggcctgctgggtaccgatgctttccaggaagccgatatccgcggcatcaccatgccagtgaccaagaataacttcatggtcaccgaccccaacgacattccacaggcattggctgaggcattccacctcgcgattactggtcgccctggccctgttctggtggatattcctaaggatgtccaaaacgctgaattggatttcgtctggccaccaaagatcgacctgccaggctaccgcccagtttctactccgcatgctcgacagattgagcaggctgtcaaactgatcggtgaagccaaaaagccagtcctttacattggcggcggcgttatcaaggctgatgcacacgaagaactgcgtgcatttgctgagtacaccggcatcccagttgtcaccaccttgatggcattgggtaccttcccagagtcccacgagctgcacatgggtatgccaggcatgcacggcaccgtgtccgctgttggcgcactgcagcgcagtgacctgctgattgctatcggttcccgcttcgacgaccgcgtcaccggtgacgttgacaccttcgcacctgatgccaagatcattcacgctgacattgatcctgccgaaatcggcaagatcaagcaggttgaggttccaatcgtgggcgatgcccgcgaggttcttgctcgtctgctggaaaccaccaaggcaagcaaggcagagaccgaggacatctccgagtgggttgattacctcaagggcctcaaggcacgtttcccacgtggctacgacgagcagccaggcgatctgctggcaccacagtttgtcattgaaaccctgtccaaggaagttggccccgacgcaatttactgcgccggcgttggccagcaccagatgtgggcagctcagttcgttgactttgaaaagccacgcacctggctcaactctggcggcctgggcaccatgggctacgcagttcctgcggctcttggagcaaaggctggcgcacctgacaaggaagtctgggctatcgacggcgacggctgtttccagatgaccaaccaggaactcaccaccgccgcagttgaaggtttccccattaagatcgcactaatcaacaacggaaacctgggcatggttcgccaatggcagaccctattctatgaaggacggtactcaaatactaaacttcgtaaccagggcgagtacatgcccgactttgttaccctttctgagggacttggctgtgttgccatccgcgtcaccaaagcggaggaagtactgccagccatccaaaaggctcgagagatcaacgaccgcccagtagtcatcgacttcatcgtcggtgaagacgcacaggtatggccaatggtgtctgctggatcatccaactccgatatccagtacgcactcggattgcgcccattctttgatggtgatgaatctgcagcagaagatcctgccgacattcacgaagccgtcagcgacattgatgccgccgttgaatcgaccgaggcataa

SEQ ID NO: 21 - DNA, 5802 bp, synthetic construct
  misc_feature 1..5802: note = pDC24 vector
  source 1..5802: mol_type = other DNA
gttcgcttgctgtccataaaaccgcccagtctagctatcgccatgtaagcccactgcaagctacctgctttctctttgcgcttgcgttttcccttgtccagatagcccagtagctgacattcatccggggtcagcaccgtttctgcggactggctttctacgtgttccgcttcctttagcagcccttgcgccctgagtgcttgcggcagcgtgaagctagcttttatcgccattcgccattcaggctgcgcaactgttgggaagggcgatcggtgcgggcctcttcgctattacgccagctggcgaaagggggatgtgctgcaaggcgattaagttgggtaacgccagggttttcccagtcacgacgttgtaaaacgacggccagtgaattcgagctcggtacccggggatcctctagagtcgacctgcaggcatgcaagcttggcgtaatcatggtcatagctgtttcctgtgtgaaattgttatccgctcacaattccacacaacatacgagccggaagcataaagtgtaaagcctggggtgcctaatgagtgagctaactcacattaattgcgttgcgctcactgcccgctttccagtcgggaaacctgtcgtgccagctgcattaatgaatcggccaacgcgcggggagaggcggtttgcgtattgggcgctcttccgcttcctcgctcactgactcgctgcgctcggtcgttcggctgcggcgagcggtatcagctcactcaaaggcggtaatacggttatccacagaatcaggggataacgcaggaaagaacatgtgagcaaaaggccagcaaaaggccaggaaccgtaaaaaggccgcgttgctggcgtttttccataggctccgcccccctgacgagcatcacaaaaatcgacgctcaagtcagaggtggcgaaacccgacaggactataaagataccaggcgtttccccctggaagctccctcgtgcgctctcctgttccgaccctgccgcttaccggatacctgtccgcctttctcccttcgggaagcgtggcgctttctcaatgctcacgctgtaggtatctcagttcggtgtaggtcgttcgctccaagctgggctgtgtgcacgaaccccccgttcagcccgaccgctgcgccttatccggtaactatcgtcttgagtccaacccggtaagacacgacttatcgccactggcagcagccactggtaacaggattagcagagcgaggtatgtaggcggtgctacagagttcttgaagtggtggcctaactacggctacactagaaggacagtatttggtatctgcgctctgctgaagccagttaccttcggaaaaagagttggtagctcttgatccggcaaacaaaccaccgctggtagcggtggtttttttgtttgcaagcagcagattacgcgcagaaaaaaaggatctcaagaagatcctttgatcttttctacggggtctgacgctcagtggaacgaaaactcacgttaagggattttggtcatgagattatcaaaaaggatcttcacctagatccttttggggtgggcgaagaactccagcatgagatccccgcgctggaggatcatccagccctgatagaaacagaagccactggagcacctcaaaaacaccatcatacactaaatcagtaagttggcagcatcacccgacgcactttgcgccgaataaatacctgtgacggaagatcacttcgcagaataaataaatcctggtgtccctgttgataccgggaagccctgggccaacttttggcgaaaatgagacgttgatcggcacgtaagaggttccaactttcaccataatgaaataagatcactaccgggcgtattttttgagttatcgagattttcaggagctgatagaaacagaagccactggagcacctcaaaaacaccatcatacactaaatcagtaagttggcagcatcacccgacgcactttgcgccgaataaatacctgtgacggaagatcacttcgcagaataaataaatcctggtgtccctgttgataccgggaagccctgggccaacttttggcgaaaatgagacgttgatcggcacgtaagaggttccaactttcaccataatgaaataagatcactaccgggcgtattttttgagttatcgagattttcaggagctctttggcatcgtctctcgcctgtcccctcagttcagtaatttcctgcatttgcctgtttccagtcggtagatattccacaaaacagcagggaagcagcgcttttccgctgcataaccctgcttcggggtcattatagcgattttttcggtatatccatcctttttcgcacgatatacaggattttgccaaagggttcgtgtagactttccttggtgtatccaacggcgtcagccgggcaggataggtgaagtaggcccacccgcgagcgggtgttccttcttcactgtcccttattcgcacctggcggtgctcaacgggaatcctgctctgcgaggctggccggctaccgccggcgtaacagatgagggcaagcggatggctgatgaaaccaagccaaccaggaagggcagcccacctatcaaggtgtactgccttccagacgaacgaagagcgattgaggaaaaggcggcggcggccggcatgagcctgtcggcctacctgctggccgtcggccagggctacaaaatcacgggcgtcgtggactatgagcacgtccgcgagggcgtcccggaaaacgattccgaagcccaacctttcatagaaggcggcggtggaatcgaaatctcgtgatggcaggttgggcgtcgcttggtcggtcatttcgaaaaaggttaggaatacggttagccatttgcctgcttttatatagttcatatgggattcacctttatgttgataagaaataaaagaaaatgccaataggatatcggcattttcttttgcgtttttatttgttaactgttaattgtccttgttcaaggatgctgtctttgacaacagatgttttcttgcctttgatgttcagcaggaagctcggcgcaaacgttgattgtttgtctgcgtagaatcctctgtttgtcatatagcttgtaatcacgacattgtttcctttcgcttgaggtacagcgaagtgtgagtaagtaaaggttacatcgttaggcggatcaagatccatttttaacacaaggccagttttgttcagcggcttgtatgggccagttaaagaattagaaacataaccaagcatgtaaatatcgttagacgtaatgccgtcaatcgtcatttttgatccgcgggagtcagtgaacaggtaccatttgccgttcattttaaagacgttcgcgcgttcaatttcatctgttactgtgttagatgcaatcagcggtttcatcacttttttcagtgtgtaatcatcgtttagctcaatcataccgagagcgccgtttgctaactcagccgtgcgttttttatcgctttgcagaagtttttgactttcttgacggaagaatgatgtgcttttgccatagtatgctttgttaaataaagattcttcgccttggtagccatcttcagttccagtgtttgcttcaaatactaagtatttgtggcctttatcttctacgtagtgaggatctctcagcgtatggttgtcgcctgagctgtagttgccttcatcgatgaactgctgtacattttgatacgtttttccgtcaccgtcaaagattgatttataatcctctacaccgttgatgttcaaagagctgtctgatgctgatacgttaacttgtgcagttgtcagtgtttgtttgccgtaatgtttaccggagaaatcagtgtagaataaacggatttttccgtcagatgtaaatgtggctgaacctgaccattcttgtgtttggtcttttaggatagaatcatttgcatcgaatttgtcgctgtctttaaagacgcggccagcgtttttccagctgtcaatagaagtttcgccgactttttgatagaacatgtaaatcgatgtgtcatccgcatttttaggatctccggctaatgcaaagacgatgtggtagccgtgatagtttgcgacagtgccgtcagcgttttgtaatggccagctgtcccaaacgtccaggccttttgcagaagagatatttttaattgtggacgaatcaaattcagaaacttgatatttttcatttttttgctgttcagggatttgcagcatatcatggcgtgtaatatgggaaatgccgtatgtttccttatatggcttttggttcgtttctttcgcaaacgcttgagttgcgcctcctgccagcagtgcggtagtaaaggttaatactgttgcttgttttgcaaactttttgatgttcatcgttcatgtctccttttttatgtactgtgttagcggtctgcttcttccagccctcctgtttgaagatggcaagttagttacgcacaataaaaaaagacctaaaatatgtaaggggtgacgccaaagtatacactttgccctttacacattttaggtcttgcctgctttatcagtaacaaacccgcgcgatttacttttcgacctcattctattagactctcgtttggattgcaactggtctattttcctcttttgtttgatagaaaatcataaaaggatttgcagactacgggcctaaagaactaaaaaatctatctgtttcttttcattctctgtattttttatagtttctgttgcatgggcataaagttgcctttttaatcacaattcagaaaatatcataatatctcatttcactaaataatagtgaacggcaggtatatgtgatgggttaaaaaggatcaccccagagtcccgctcagaagaactcgtcaagaaggcgatagaaggcgatgcgctgcgaatcgggagcggcgataccgtaaagcacgaggaagcggtcagcccattcgccgccaagctcttcagcaatatcacgggtagccaacgctatgtcctgatagcggtccgccacacccagccggccacagtcgatgaatccagaaaagcggccattttccaccatgatattcggcaagcaggcatcgccatgggtcacgacgagatcctcgccgtcgggcatccgcgccttgagcctggcgaacagttcggctggcgcgagcccctgatgctcttcgtccagatcatcctgatcgacaagaccggcttccatccgagtacgtgctcgctcgatgcgatgtttcgcttggtggtcgaatgggcaggtagccggatcaagcgtatgcagccgccgcattgcatcagccatgatggatactttctcggcaggagcaaggtgagatgacaggagatcctgccccggcacttcgcccaatagcagccagtcccttcccgcttcagtgacaacgtcgagacagctgcgcaaggaacgcccgtcgtggccagccacgatagccgcgctgcctcgtcttggagttcattcagggcaccggacaggtcggtcttgacaaaaagaaccgggcgcccctgcgctgacagccggaacacggcggcatcagagcagccgattgtctgttgtgcccagtcatagccgaatagcctctccacccaagcggccggagaacctgcgtgcaatccatcttgttcaatcatgcgaaacgatcctcatcctgtctcttgatcagatcttgatcccctgcgccatcagatccttggcggcaagaaagccatccagtttactttgcagggcttcccaaccttaccagagggcgccccagctggcaattccg